European Patent Application EP 4 286 411 A1, published December 6, 2023. Title: HUMANIZED ANTIBODY AGAINST TNFR2 AND USE THEREOF. Applicant: SHANDONG SIMCERE BIOPHARMACEUTICAL CO., LTD. The sequence listing filed with the application follows.

SEQUENCE LISTING (43 sequences)

SEQ ID NO: 1 - protein, 5 aa, Artificial sequence
  Obtained by synthesis
TYDLS

SEQ ID NO: 2 - protein, 17 aa, Artificial sequence
  Obtained by synthesis
YINNGGISTYYSDTVKG

SEQ ID NO: 3 - protein, 12 aa, Artificial sequence
  Obtained by synthesis
GPFYGSANYFDY

SEQ ID NO: 4 - protein, 11 aa, Artificial sequence
  Obtained by synthesis
RTSESIYSNLP

SEQ ID NO: 5 - protein, 7 aa, Artificial sequence
  Obtained by synthesis
DATKLAE

SEQ ID NO: 6 - protein, 9 aa, Artificial sequence
  Obtained by synthesis
QHFWVTPWT

SEQ ID NO: 7 - protein, 5 aa, Artificial sequence
  Obtained by synthesis
NYWMN

SEQ ID NO: 8 - protein, 17 aa, Artificial sequence
  Obtained by synthesis
MIHPSDTETRLNQNFKD

SEQ ID NO: 9 - protein, 14 aa, Artificial sequence
  Obtained by synthesis
GEGLGAARSVSMDY

SEQ ID NO: 10 - protein, 11 aa, Artificial sequence
  Obtained by synthesis
RASQDISNYLN

SEQ ID NO: 11 - protein, 7 aa, Artificial sequence
  Obtained by synthesis
YTAILHS

SEQ ID NO: 12 - protein, 9 aa, Artificial sequence
  Obtained by synthesis
QQGNTLPWT

SEQ ID NO: 13 - protein, 5 aa, Artificial sequence
  Obtained by synthesis
DIYMH

SEQ ID NO: 14 - protein, 17 aa, Artificial sequence
  Obtained by synthesis
RIDPATGNTKHDPKFQD

SEQ ID NO: 15 - protein, 11 aa, Artificial sequence
  Obtained by synthesis
SPYGDFGAMDY

SEQ ID NO: 16 - protein, 12 aa, Artificial sequence
  Obtained by synthesis
TASSSVSSNYLH

SEQ ID NO: 17 - protein, 7 aa, Artificial sequence
  Obtained by synthesis
STSNLPS

SEQ ID NO: 18 - protein, 9 aa, Artificial sequence
  Obtained by synthesis
HQYHRSPWT

SEQ ID NO: 19 - protein, 121 aa, Artificial sequence
  Obtained by synthesis
EVQLVESGGGLVQPGGSLRLSCAASGFAFSTYDLSWVRQAPGKGLEWVAYINNGGISTYYSDTVKGRFTISRDNAKNTLYLQMNSLRAEDTAVYYCVRGPFYGSANYFDYWGQGTLVTVSS

SEQ ID NO: 20 - protein, 121 aa, Artificial sequence
  Obtained by synthesis
EVQLVESGGGLVQPGGSLRLSCAASGFAFSTYDLSWVRQAPGKGLEWVAYINNGGISTYYSDTVKGRFTISRDNAKNSLYLQMNSLRAEDTAVYYCVRGPFYGSANYFDYWGQGTLVTVSS

SEQ ID NO: 21 - protein, 123 aa, Artificial sequence
  Obtained by synthesis
QVQLVQSGAEVKKPGASVKVSCKASGYSFTNYWMNWVRQAPGQRLEWMGMIHPSDTETRLNQNFKDRVTITRDTSASTAYMELSSLRSEDTAVYYCARGEGLGAARSVSMDYWGQGTLVTVSS

SEQ ID NO: 22 - protein, 123 aa, Artificial sequence
  Obtained by synthesis
QVQLVQSGAEVKKPGSSVKVSCKASGYSFTNYWMNWVRQAPGQGLEWMGMIHPSDTETRLNQNFKDKATITADKSTSTAYMELSSLRSEDTAVYYCARGEGLGAARSVSMDYWGQGTLVTVSS

SEQ ID NO: 23 - protein, 123 aa, Artificial sequence
  Obtained by synthesis
QVQLVQSGAEVKKPGSSVKVSCKASGYSFTNYWMNWVRQAPGQGLEWMGMIHPSDTETRLNQNFKDRVTITADKSTSTAYMELSSLRSEDTAVYYCARGEGLGAARSVSMDYWGQGTLVTVSS

SEQ ID NO: 24 - protein, 123 aa, Artificial sequence
  Obtained by synthesis
QVQLVQSGAEVKKPGSSVKVSCKASGYSFTNYWMNWVKQAPGQGLEWIGMIHPSDTETRLNQNFKDKATLTVDKSTSTAYMELSSLRSEDTAVYYCARGEGLGAARSVSMDYWGQGTLVTVSS

SEQ ID NO: 25 - protein, 123 aa, Artificial sequence
  Obtained by synthesis
QVQLVQSGAEVKKPGSSVKVSCKASGYSFTNYWMNWVRQAPGQGLEWMGMIHPSDTETRLNQNFKDRVTITVDKSTSTAYMELSSLRSEDTAVYYCARGEGLGAARSVSMDYWGQGTLVTVSS

SEQ ID NO: 26 - protein, 120 aa, Artificial sequence
  Obtained by synthesis
QVQLVQSGAEVKKPGASVKVSCKASGFNNKDIYMHWVRQAPGQGLEWIGRIDPATGNTKHDPKFQDRVTMTSDTSTNTVYMELSSLRSEDTAVYYCARSPYGDFGAMDYWGQGTLVTVSS

SEQ ID NO: 27 - protein, 120 aa, Artificial sequence
  Obtained by synthesis
QVQLVQSGSELKKPGASVKVSCKASGFNNKDIYMHWVRQAPGQGLEWMGRIDPATGNTKHDPKFQDKAVLSSDTSVSTAYLQISSLKAEDTAVYYCARSPYGDFGAMDYWGQGTLVTVSS

SEQ ID NO: 28 - protein, 107 aa, Artificial sequence
  Obtained by synthesis
DIQMTQSPSSLSASVGDRVTITCRTSESIYSNLPWYQQKPGKAPKLLLYDATKLAEGVPSRFSGSGSGTDYTLTISSLQPEDFATYYCQHFWVTPWTFGQGTKVEIK

SEQ ID NO: 29 - protein, 107 aa, Artificial sequence
  Obtained by synthesis
DIQMTQSPSSLSASVGDRVTITCRTSESIYSNLPWYQQKPGKSPKLLIYDATKLAEGVPSRFSGSGSGTDFTLTISSLQPEDFATYYCQHFWVTPWTFGQGTKVEIK

SEQ ID NO: 30 - protein, 107 aa, Artificial sequence
  Obtained by synthesis
DIQMTQSPSSLSASVGDRVTITCRTSESIYSNLPWYQQKPGKAPKLLIYDATKLAEGVPSRFSGSGSGTDYTLTISSLQPEDFATYYCQHFWVTPWTFGQGTKVEIK

SEQ ID NO: 31 - protein, 107 aa, Artificial sequence
  Obtained by synthesis
DIQMTQSPSSLSASVGDRVTITCRTSESIYSNLPWYQQKPGKSPKLLVYDATKLAEGVPSRFSGSGSGTDYTLTISSLQPEDFATYYCQHFWVTPWTFGQGTKVEIK

SEQ ID NO: 32 - protein, 107 aa, Artificial sequence
  Obtained by synthesis
DIQMTQSPSSLSASVGDRVTITCRASQDISNYLNWYQQKPDGTVKLLIYYTAILHSGVPSRFSGSGSGTDYSLTISSLQPEDFATYFCQQGNTLPWTFGQGTKVEIK

SEQ ID NO: 33 - protein, 108 aa, Artificial sequence
  Obtained by synthesis
DIQMTQSPSSLSASVGDRVTITCTASSSVSSNYLHWYQQKPGKAPKLWIYSTSNLPSGVPSRFSGSGSGTDFTLTISSLQPEDFATYYCHQYHRSPWTFGQGTKVEIK

SEQ ID NO: 34 - protein, 108 aa, Artificial sequence
  Obtained by synthesis
DIQMTQSPSSLSASVGDRVTITCTASSSVSSNYLHWYQQKPGSSPKLWIYSTSNLPSGVPSRFSGSGSGTDFTLTISSLQPEDFATYYCHQYHRSPWTFGQGTKVEIK

SEQ ID NO: 35 - protein, 108 aa, Artificial sequence
  Obtained by synthesis
DIQMTQSPSSLSASVGDRVTITCTASSSVSSNYLHWYQQKPGKAPKLLIYSTSNLPSGVPSRFSGSGSGTDFTLTISSLQAEDAATYYCHQYHRSPWTFGQGTKVEIK

SEQ ID NO: 36 - protein, 108 aa, Artificial sequence
  Obtained by synthesis
DIQMTQSPSSLSASVGDRVTITCTASSSVSSNYLHWYQQKPGKAPKLLIYSTSNLPSGVPSRFSGSGSGTDYSLTISSLQPEDFATYYCHQYHRSPWTFGQGTKVEIK

SEQ ID NO: 37 - protein, 108 aa, Artificial sequence
  Obtained by synthesis
DIQMTQSPSSLSASVGDRVTITCTASSSVSSNYLHWYQQKPGKAPKLLIYSTSNLPSGVPSRFSGSGSGTDFTLTISSLQPEDFATYYCHQYHRSPWTFGQGTKVEIK

SEQ ID NO: 38 - protein, 121 aa, Artificial sequence
  Obtained by synthesis
EVQLQESGGGLVQPGGSLNLSCAASGFAFSTYDLSWVRQTPEKRLEWVAYINNGGISTYYSDTVKGRFTISRDNAKNTLYLQMSSLKSEDTAMYYCVRGPFYGSANYFDYWGQGTTVTVSS

SEQ ID NO: 39 - protein, 107 aa, Artificial sequence
  Obtained by synthesis
EIVMTQSPASLSLSVGETVTITCRTSESIYSNLPWYQQKQGKSPQLLVYDATKLAEGVPSRFSGSESGTQYSLKINSLQSEDFGTYYCQHFWVTPWTFGGGTKLEIK

SEQ ID NO: 40 - protein, 123 aa, Artificial sequence
  Obtained by synthesis
EVQLQESGAELVRPGASVKLSCKASGYSFTNYWMNWVKQRPGQGLEWIGMIHPSDTETRLNQNFKDKATLTVDKSSSTSYMQLSSPTSEDSAVYYCARGEGLGAARSVSMDYWGQGTTVTVSS

SEQ ID NO: 41 - protein, 107 aa, Artificial sequence
  Obtained by synthesis
DILMTQSPSSLSASLGDRVTISCRASQDISNYLNWYQQKPDGTVKVLIYYTAILHSGVPSRFSGSGSGTDYSLTISNLEQEDIATYFCQQGNTLPWTFGGGTKLEIK

SEQ ID NO: 42 - protein, 120 aa, Artificial sequence
  Obtained by synthesis
EVQLQESGPEIVKPGASVKLSCTASGFNNKDIYMHWVKQRPEQGLEWIGRIDPATGNTKHDPKFQDKATLSSDTSSNTAYLQFSSLTSEDTAVYYCAHSPYGDFGAMDYWGQGTTVTVSS

SEQ ID NO: 43 - protein, 108 aa, Artificial sequence
  Obtained by synthesis
DIQMTQSPAIMSASLGERVTMTCTASSSVSSNYLHWYQQKPGSSPKLWIYSTSNLPSGVPARFSGSGSGTSYSLTISSMEAEDAATYYCHQYHRSPWTFGGGTKLEIK